European Patent Application EP 4 729 536 A1, published April 22, 2026. Title: 乙肝病毒表面抗体及其应用. Applicant: 复旦大学. Application WO. The sequence listing filed with the application follows.

SEQUENCE LISTING (497 sequences)

SEQ ID NO: 1 - protein, 123 aa, synthetic construct
QVQMVQSGAEVKKPGSSVKVSCKASGGAFGRYAVSWLRQAPGQGLEWMGRIIPLLGIVDYAQKFQGRVTISAHRSTGTAYMELSSLRSEDTALFFCAREGNDGVVVPYFFESWGQGTLVTVSS

SEQ ID NO: 2 - protein, 8 aa, synthetic construct
GGAFGRYA

SEQ ID NO: 3 - protein, 8 aa, synthetic construct
IIPLLGIV

SEQ ID NO: 4 - protein, 16 aa, synthetic construct
AREGNDGVVVPYFFES

SEQ ID NO: 5 - protein, 108 aa, synthetic construct
EIVLTQSPGTLSVSPGERATLSCRASQSVSRNYLVWYQQKPGQPPKLLIYGASSRATGVPDRFSGSGSGTDFTLTINRLVPEDFAVYFCQQYGSSPITFGGGTKLEIK

SEQ ID NO: 6 - protein, 7 aa, synthetic construct
QSVSRNY

SEQ ID NO: 7 - skipped

SEQ ID NO: 8 - protein, 9 aa, synthetic construct
QQYGSSPIT

SEQ ID NO: 9 - protein, 121 aa, synthetic construct
QVQLVQSGPEVKMPGSSVRVSCKASGGTFRSHTFSWVRQAPGQGLEWVGRVLPVLRVANYAQKLQGRVTITADKSTLTTYMDLSSLRSDDTAVYYCARQGEKSHLDAFDIWGQGTMVIVSS

SEQ ID NO: 10 - protein, 8 aa, synthetic construct
GGTFRSHT

SEQ ID NO: 11 - protein, 8 aa, synthetic construct
VLPVLRVA

SEQ ID NO: 12 - protein, 14 aa, synthetic construct
ARQGEKSHLDAFDI

SEQ ID NO: 13 - protein, 107 aa, synthetic construct
DIQMTQSPSSLSASVGDRVTITCRASQDIRDFLAWFQQKPGKAPKSLIFATSSLHSGVPSKFSGSGSGTYFTLTISSLQPEDIATYYCQQYINYPPTFGGGTKVEIK

SEQ ID NO: 14 - protein, 6 aa, synthetic construct
QDIRDF

SEQ ID NO: 15 - skipped

SEQ ID NO: 16 - protein, 9 aa, synthetic construct
QQYINYPPT

SEQ ID NO: 17 - protein, 119 aa, synthetic construct
QVQLVQSGAEVKRPGSSVKVSCRTSGGSFSREGLSWVRQAPGQGLEWMGRIIPIVGIVDYAQKFQGRVTITADKSTSTGYIEVRRLTSEDTAMYYCAKDSGYSGHSQPWGQGTLVTVSS

SEQ ID NO: 18 - protein, 8 aa, synthetic construct
GGSFSREG

SEQ ID NO: 19 - protein, 8 aa, synthetic construct
IIPIVGIV

SEQ ID NO: 20 - protein, 12 aa, synthetic construct
AKDSGYSGHSQP

SEQ ID NO: 21 - protein, 107 aa, synthetic construct
DIQMTQSPSSLSASVGDRVTITCRASQTISIFLAWFQQKPGQAPKLLIYKASSLQSGVPSRFSGSGSGTDFTLTITSLQPDDFATYYCQQSDRVPWTFGQGTKVEMK

SEQ ID NO: 22 - protein, 6 aa, synthetic construct
QTISIF

SEQ ID NO: 23 - skipped

SEQ ID NO: 24 - protein, 9 aa, synthetic construct
QQSDRVPWT

SEQ ID NO: 25 - protein, 126 aa, synthetic construct
EVQLSESGGGLVQPGGSLRLSCAASGLTLSNPPMNWVRQAPGKGLEWVSVIYGGGNTLYADSVKGRFSVSRDNSKNTVYLQMHSLRVDDTAVYYCAKEGSAVRGVISLEAYGMDVWGPGTTVIVAS

SEQ ID NO: 26 - protein, 8 aa, synthetic construct
GLTLSNPP

SEQ ID NO: 27 - protein, 7 aa, synthetic construct
IYGGGNT

SEQ ID NO: 28 - protein, 20 aa, synthetic construct
AKEGSAVRGVISLEAYGMDV

SEQ ID NO: 29 - protein, 109 aa, synthetic construct
EIVLTQSPRTLSLSPGERATLSCRASQSFSSGYLAWYQQKPGQAPRLLIYGASTRAPGIPHRFSGSGSGTDFTLTISRVEPEDFVVYYCQQYGSSPPFSFGPGTKVDFK

SEQ ID NO: 30 - protein, 7 aa, synthetic construct
QSFSSGY

SEQ ID NO: 31 - skipped

SEQ ID NO: 32 - protein, 10 aa, synthetic construct
QQYGSSPPFS

SEQ ID NO: 33 - protein, 123 aa, synthetic construct
QGPLVQSGAEMRKPGASVKVSCKASGYIFDKYGFTWVRQAPGQGLEWMGWISANNGNTKYAPRLQGRVTMTTDSSTSTGYLELRSLRSDDTAVYYCARGLSAIRVGPLGFDFWGQGTLVTVSS

SEQ ID NO: 34 - protein, 8 aa, synthetic construct
GYIFDKYG

SEQ ID NO: 35 - protein, 8 aa, synthetic construct
ISANNGNT

SEQ ID NO: 36 - protein, 16 aa, synthetic construct
ARGLSAIRVGPLGFDF

SEQ ID NO: 37 - protein, 110 aa, synthetic construct
QSALTQSRSVSGSPGQSVTISCTGTRTDVGGYNYVSWYQQHPGTAPKLIIYDVSNRPSGVPERFSGSKSGNTASLTISGLQAEDEADYYCCSYAGTNTWVFGGGTKLTVR

SEQ ID NO: 38 - protein, 9 aa, synthetic construct
RTDVGGYNY

SEQ ID NO: 39 - skipped

SEQ ID NO: 40 - protein, 10 aa, synthetic construct
CSYAGTNTWV

SEQ ID NO: 41 - protein, 120 aa, synthetic construct
QVQLVQSGAEVKKPGYSVKVSCKASEGTFGRNTINWLRQVPGHGPEWMGSIIPILGTPFYAQKFQGRVTISADKFTGTAYMELTRLTSQDTAVYYCAKEMSSGYSCLDVWGQGTTVTVSS

SEQ ID NO: 42 - protein, 8 aa, synthetic construct
EGTFGRNT

SEQ ID NO: 43 - protein, 8 aa, synthetic construct
IIPILGTP

SEQ ID NO: 44 - protein, 13 aa, synthetic construct
AKEMSSGYSCLDV

SEQ ID NO: 45 - protein, 108 aa, synthetic construct
EVVLTQSPGTLSLSPGDRATLSCRASQSVNTAYLAWYQQKPGQTPRLLVFGTSSRATGIPDRFSGSGSGTDFTLTISRLEPEDFAVYYCQQYGNSPLTFGGGTKVEIK

SEQ ID NO: 46 - protein, 7 aa, synthetic construct
QSVNTAY

SEQ ID NO: 47 - skipped

SEQ ID NO: 48 - protein, 9 aa, synthetic construct
QQYGNSPLT

SEQ ID NO: 49 - protein, 119 aa, synthetic construct
QVQLVQSGTEVKKPGSSVKVSCEASGGLSRSHAFNWVRQAPGQGLEWVGRILPFLSITNYAQYLQGRVTITADRSITKTYLELRGLRSQDTAVYFCATELSGSTNLDYWGQGTLVTVSS

SEQ ID NO: 50 - protein, 8 aa, synthetic construct
GGLSRSHA

SEQ ID NO: 51 - protein, 8 aa, synthetic construct
ILPFLSIT

SEQ ID NO: 52 - protein, 12 aa, synthetic construct
ATELSGSTNLDY

SEQ ID NO: 53 - protein, 111 aa, synthetic construct
QSVLTQPPSVSGAPGQRVTISCSGSSSNIGAGSDVHWYQQFPGTAPKLLIYRNNNRPSGVPDRFSGSKSGSSASLAITGLQAEDEAAYYCQSFDRSLSASVFGGGTKLTVL

SEQ ID NO: 54 - protein, 9 aa, synthetic construct
SSNIGAGSD

SEQ ID NO: 55 - skipped

SEQ ID NO: 56 - protein, 11 aa, synthetic construct
QSFDRSLSASV

SEQ ID NO: 57 - protein, 121 aa, synthetic construct
QAQLVQSGAEVKTPGSSVKVSCKASGGTFMRQALSWVRQAPGQSLEWMGSIIPMLYKTTYAQKFQGRLTITADRSRTTVYMELSSLRSEDTAIYYCARDPSVATSEDFDYWGLGTQVTVPS

SEQ ID NO: 58 - protein, 8 aa, synthetic construct
GGTFMRQA

SEQ ID NO: 59 - protein, 8 aa, synthetic construct
IIPMLYKT

SEQ ID NO: 60 - protein, 14 aa, synthetic construct
ARDPSVATSEDFDY

SEQ ID NO: 61 - protein, 111 aa, synthetic construct
QVVLTQSPSASASLGASVKLTCTLSSGHSNFPIAWHQQQPEKGPRYLMKVNSDGSHNKGDGIPDRFSGSSSGAERYLTISSLQSEDEADYYCQTWGTGFQVFGGGTKLSVL

SEQ ID NO: 62 - protein, 7 aa, synthetic construct
SGHSNFP

SEQ ID NO: 63 - protein, 7 aa, synthetic construct
VNSDGSH

SEQ ID NO: 64 - protein, 9 aa, synthetic construct
QTWGTGFQV

SEQ ID NO: 65 - protein, 116 aa, synthetic construct
QVQLVQSGAEVKKPGSSVKVSCKASGGTFSRDAISWVRQAPGQGLEWMGRILPIVGITDYSRKFQGRVTITADKSTSTAYMALSSLRSEDTATYFCAGDPGYISNWGQGTLVTVSS

SEQ ID NO: 66 - protein, 8 aa, synthetic construct
GGTFSRDA

SEQ ID NO: 67 - protein, 8 aa, synthetic construct
ILPIVGIT

SEQ ID NO: 68 - protein, 9 aa, synthetic construct
AGDPGYISN

SEQ ID NO: 69 - protein, 107 aa, synthetic construct
DIQMTQSPSSLSASVGDRVTITCRASQSISVYLSWYQQKPGKVPNLLIYAASSLQTGVPSRFSGSGSGTDFTLTISSLEPEDYATYFCLQSDRPPWTFAQGTKVEIK

SEQ ID NO: 70 - protein, 6 aa, synthetic construct
QSISVY

SEQ ID NO: 71 - skipped

SEQ ID NO: 72 - protein, 9 aa, synthetic construct
LQSDRPPWT

SEQ ID NO: 73 - protein, 119 aa, synthetic construct
QVQLVQSGSEVKKPGSSVKVSCKASGDTVRGSPINWLRQAPGQGLEWMGRIIPLLRVVDYAHSFQGRLTITADKSTKTAYMDLSRLRSDDTAVYYCATDEGSTYYFDSWGQGTLVTVSS

SEQ ID NO: 74 - protein, 8 aa, synthetic construct
GDTVRGSP

SEQ ID NO: 75 - protein, 8 aa, synthetic construct
IIPLLRVV

SEQ ID NO: 76 - protein, 12 aa, synthetic construct
ATDEGSTYYFDS

SEQ ID NO: 77 - protein, 107 aa, synthetic construct
DIQMTQSPSSLSASVGDRVSITCRASQSVSRHFNWYRQKPGKAPELLIFAASSLQSGVPSRFSGSGSGTDFTLTISNLQPEDFATYYCQQSYRTPPTFGQGTKVEIK

SEQ ID NO: 78 - protein, 6 aa, synthetic construct
QSVSRH

SEQ ID NO: 79 - skipped

SEQ ID NO: 80 - protein, 9 aa, synthetic construct
QQSYRTPPT

SEQ ID NO: 81 - protein, 118 aa, synthetic construct
QVQLVQSGAEVKKPGSSVKVSCKASGGTFFRDAVSWLRQAPGQGPEWMGRIIPVLRVVDYAQKFQGRVTITADKSTSTVYLGLSSLRSDDTALYYCARDPGYSDDPRWGQGTLVTVSS

SEQ ID NO: 82 - protein, 8 aa, synthetic construct
GGTFFRDA

SEQ ID NO: 83 - protein, 8 aa, synthetic construct
IIPVLRVV

SEQ ID NO: 84 - protein, 11 aa, synthetic construct
ARDPGYSDDPR

SEQ ID NO: 85 - protein, 108 aa, synthetic construct
EIVLTQSPGTLSLSPGERATLSCRASQSISSAYFAWFQQKPGQVPRLLISGASSRATGIPDRFSGSGSGTEFTLTINRLEPEDFAVYYCLQYGNSPWTFGQGTKVEIK

SEQ ID NO: 86 - protein, 7 aa, synthetic construct
QSISSAY

SEQ ID NO: 87 - skipped

SEQ ID NO: 88 - protein, 9 aa, synthetic construct
LQYGNSPWT

SEQ ID NO: 89 - protein, 116 aa, synthetic construct
QVQLVQSGAEVKKPGSSVTVSCKASGGSVSRFPINWVRQAPGQGLEWMGRIIPLLGVVDYAQRFQGRATISADKFTGTISMQLRSLRLEDTAVFYCARELDAFDIWGRGTMVTVSL

SEQ ID NO: 90 - protein, 8 aa, synthetic construct
GGSVSRFP

SEQ ID NO: 91 - protein, 8 aa, synthetic construct
IIPLLGVV

SEQ ID NO: 92 - protein, 9 aa, synthetic construct
ARELDAFDI

SEQ ID NO: 93 - protein, 108 aa, synthetic construct
EIVLTQSPGTLSLSPGERATLSCRASQTVSNAYFAWYQQKPGQAPRLLIYGASSRATGIPDRFSGSGSGTDFTLTISRLEPEDFAVYYCLQFGSSPATFGQGTKVEIK

SEQ ID NO: 94 - protein, 7 aa, synthetic construct
QTVSNAY

SEQ ID NO: 95 - skipped

SEQ ID NO: 96 - protein, 9 aa, synthetic construct
LQFGSSPAT

SEQ ID NO: 97 - protein, 121 aa, synthetic construct
QVQLVQSGPEVKKPGSSVKVSCKASGGTFNRDTFNWVRQAPGQGLEWMGGIIPIIPITNYAQRFRGRVKIYADKSTTTIYMDLSSLRSEDTAVYYCAYSQGGNSDWYYDLWGRGTLVTVSS

SEQ ID NO: 98 - protein, 8 aa, synthetic construct
GGTFNRDT

SEQ ID NO: 99 - protein, 8 aa, synthetic construct
IIPIIPIT

SEQ ID NO: 100 - protein, 14 aa, synthetic construct
AYSQGGNSDWYYDL

SEQ ID NO: 101 - protein, 108 aa, synthetic construct
EIVLTQSPGTLSLSPGESATVSCRASQSVSSNYLAWYQQRPGQASRLLIYGASSRATGIPDRFSGSGSGTDFTLTINRLEPEDFAVYFCQQYGSSPQTFGQGTKVEIK

SEQ ID NO: 102 - protein, 7 aa, synthetic construct
QSVSSNY

SEQ ID NO: 103 - skipped

SEQ ID NO: 104 - protein, 9 aa, synthetic construct
QQYGSSPQT

SEQ ID NO: 105 - protein, 120 aa, synthetic construct
QVQLVQSGSEVKKPGHSVKVSCKASGGTFSRDNINWVRQAPGQGLEWMGMTIPILRIANYAQKFQDRLTITADKFTGTVYMELRSLRSDDTAVYYCAKDMSSGYSCLDVWGQGTTVTVST

SEQ ID NO: 106 - protein, 8 aa, synthetic construct
GGTFSRDN

SEQ ID NO: 107 - protein, 8 aa, synthetic construct
TIPILRIA

SEQ ID NO: 108 - protein, 13 aa, synthetic construct
AKDMSSGYSCLDV

SEQ ID NO: 109 - protein, 108 aa, synthetic construct
EIVLTQSPGTLSLSPGERATLSCRASQSVPTGHFAWYQQKPGQAPRLLIFGASSRATGIPDRFSGSGSGTVFTLTISKLEPEDFAVYYCQQFGSSPLTFGGGTRVEIK

SEQ ID NO: 110 - protein, 7 aa, synthetic construct
QSVPTGH

SEQ ID NO: 111 - skipped

SEQ ID NO: 112 - protein, 9 aa, synthetic construct
QQFGSSPLT

SEQ ID NO: 113 - protein, 117 aa, synthetic construct
LVQLVQSGAEVKKPGSSVKVSCKASGGTFGRNAVSWVRQAPGQGLEWMGRIIPLLGIGENAPKFQGRVTITADKFTGTVYMALSSLRSEDTAVYFCARESPDAFDIWGQGTMVTVSS

SEQ ID NO: 114 - protein, 8 aa, synthetic construct
GGTFGRNA

SEQ ID NO: 115 - protein, 8 aa, synthetic construct
IIPLLGIG

SEQ ID NO: 116 - protein, 10 aa, synthetic construct
ARESPDAFDI

SEQ ID NO: 117 - protein, 107 aa, synthetic construct
EIVLTQSPGTLSLSPGERATLSCRASQPASGIIAWYQRKPGQAPRLLIYGASSRATGIPDRFSGSGSGTDFTLTISRLEPDDFAVYYCHQYRIAPYTFGQGTKVEIK

SEQ ID NO: 118 - protein, 6 aa, synthetic construct
QPASGI

SEQ ID NO: 119 - skipped

SEQ ID NO: 120 - protein, 9 aa, synthetic construct
HQYRIAPYT

SEQ ID NO: 121 - protein, 128 aa, synthetic construct
QVQLVESGGGVVHPGRSLRLSCKASGFTFNSHGMHWVRKAPGKGLEWVAFIWDDGSNKFYGDSVKGRFTISRDNSKNTLYLQMNSLRAEDTAVYYCASRPNVGYYRTSYGYYYGMDLWGRGTTVTVSS

SEQ ID NO: 122 - protein, 8 aa, synthetic construct
GFTFNSHG

SEQ ID NO: 123 - protein, 8 aa, synthetic construct
IWDDGSNK

SEQ ID NO: 124 - protein, 21 aa, synthetic construct
ASRPNVGYYRTSYGYYYGMDL

SEQ ID NO: 125 - protein, 112 aa, synthetic construct
DIVMTQSPLSLTVTPGEPASISCRSSQSLFHTNGHKYLDWHVQKPGQSPQLLIYLGSSRASGVPDRFSGSGSGTDFTLKISRVEAEDVGIYYCMQTLQTPITFGQGTRLEIK

SEQ ID NO: 126 - protein, 11 aa, synthetic construct
QSLFHTNGHKY

SEQ ID NO: 127 - skipped

SEQ ID NO: 128 - protein, 9 aa, synthetic construct
MQTLQTPIT

SEQ ID NO: 129 - protein, 119 aa, synthetic construct
QVQLVQSGAEVKKPGSSLKVSCKPSGGTLSNYGFSWVRQAPGQGLDWMGRILPIIGIVNYAQKFRGRVRITADKSTNTAFMELSSLRSEDTAVYFCARDAGGGNAFDIWGQGTIVTVSS

SEQ ID NO: 130 - protein, 8 aa, synthetic construct
GGTLSNYG

SEQ ID NO: 131 - protein, 8 aa, synthetic construct
ILPIIGIV

SEQ ID NO: 132 - protein, 12 aa, synthetic construct
ARDAGGGNAFDI

SEQ ID NO: 133 - protein, 106 aa, synthetic construct
SYELIQPPSLSVSPGQTASITCSGDTLAYKHTSWYQQKPGQSPVVVIYQHTKRPSGIPERFSGSKSGNTATLTISGTQAMDEADYYCQAWDSSTAIFGGGTKLTVL

SEQ ID NO: 134 - protein, 6 aa, synthetic construct
TLAYKH

SEQ ID NO: 135 - skipped

SEQ ID NO: 136 - protein, 9 aa, synthetic construct
QAWDSSTAI

SEQ ID NO: 137 - protein, 124 aa, synthetic construct
QITLKESGPTLVKPTQTLTLTCSFSGFSLSTFGVGVGWIRQPPRKAPEWLAVIYWDDDKRYSPSLKNRLTITKDTSNRQVVLTLTNMAPVDTATYYCTYIPGMASTGTPWFDPWGQGTLVTVSS

SEQ ID NO: 138 - protein, 10 aa, synthetic construct
GFSLSTFGVG

SEQ ID NO: 139 - protein, 7 aa, synthetic construct
IYWDDDK

SEQ ID NO: 140 - protein, 16 aa, synthetic construct
TYIPGMASTGTPWFDP

SEQ ID NO: 141 - protein, 110 aa, synthetic construct
QSVLTQPPSASGTPGQRVTISCSGSRSNIGSNTVNWYQQLPGAAPKVLIYSTNQRPSGFPDRFSGSKSGTSASLAIRGLQSEDEADYYCSTWDDSLNGVVFGGGTKLTVL

SEQ ID NO: 142 - protein, 8 aa, synthetic construct
RSNIGSNT

SEQ ID NO: 143 - skipped

SEQ ID NO: 144 - protein, 11 aa, synthetic construct
STWDDSLNGVV

SEQ ID NO: 145 - protein, 122 aa, synthetic construct
QVQLVQSGAEVKKPGASVRVSCRASGYTFTGHAIHWVRQAPGHGLECMGWTNIRSGNTRYSANFQGKVTMTRDTSARTAYMDLSSLRFEDTAVYFCAREAYTGAVFDAFDLWGQGTLVTVSS

SEQ ID NO: 146 - protein, 8 aa, synthetic construct
GYTFTGHA

SEQ ID NO: 147 - protein, 8 aa, synthetic construct
TNIRSGNT

SEQ ID NO: 148 - protein, 15 aa, synthetic construct
AREAYTGAVFDAFDL

SEQ ID NO: 149 - protein, 108 aa, synthetic construct
DIQMTQFPSTLSASVGDRVTITCRASQSISGWLAWYQQRPGKAPKLLIYQASKLEGGVPSRFSGSGSGTDYTLTISNLQPEDSATYYCQRYNSYSSWTFGQGTKVDIK

SEQ ID NO: 150 - protein, 6 aa, synthetic construct
QSISGW

SEQ ID NO: 151 - skipped

SEQ ID NO: 152 - protein, 10 aa, synthetic construct
QRYNSYSSWT

SEQ ID NO: 153 - protein, 115 aa, synthetic construct
EVQLAESGGGLVRPGGSLRLSCAASGFTFSNYNFNWVRQAPGKGLEWVASISGGSLNIYYADSVKGRFTISRDDPKDSLYLQMNSLRHEDTAVYYCARTFYFDFWGQGTLVTVSS

SEQ ID NO: 154 - protein, 8 aa, synthetic construct
GFTFSNYN

SEQ ID NO: 155 - protein, 8 aa, synthetic construct
ISGGSLNI

SEQ ID NO: 156 - protein, 8 aa, synthetic construct
ARTFYFDF

SEQ ID NO: 157 - protein, 108 aa, synthetic construct
EIVMTQSPATLSVSPGERATLACRASQSVRSNLAWYQEKPGQAPRLLIYSTSTRATGIPARFSGRGYGTEFTLTISSLQPEDSAVYYCHQYDIWPPDTFGQGTKLEVK

SEQ ID NO: 158 - protein, 6 aa, synthetic construct
QSVRSN

SEQ ID NO: 159 - skipped

SEQ ID NO: 160 - protein, 10 aa, synthetic construct
HQYDIWPPDT

SEQ ID NO: 161 - protein, 120 aa, synthetic construct
QVQLVQSGAEVRKPGSSVKVSCKVSGGSFTNYIITWVRQAPGQGFQWMGRIIPSLNVANYAQKFQGRVSISADKSTATVYMELTGLTSDDTAVFYCARDGLYNWKDGVHWGQGTLVTVSS

SEQ ID NO: 162 - protein, 8 aa, synthetic construct
GGSFTNYI

SEQ ID NO: 163 - protein, 8 aa, synthetic construct
IIPSLNVA

SEQ ID NO: 164 - protein, 13 aa, synthetic construct
ARDGLYNWKDGVH

SEQ ID NO: 165 - protein, 113 aa, synthetic construct
DIVLTQTPRALSVTPGQPASMSCKSSQSLLHTDGKTYLYWFLQRPGQPPQLLISEVSTRFSGVPDRVSGSGSGTDFTLKISRVEAEDVGVYFCMQGIHHPPWTFGQGTKVEIK

SEQ ID NO: 166 - protein, 11 aa, synthetic construct
QSLLHTDGKTY

SEQ ID NO: 167 - skipped

SEQ ID NO: 168 - protein, 10 aa, synthetic construct
MQGIHHPPWT

SEQ ID NO: 169 - protein, 125 aa, synthetic construct
EGQLVESGGGVIQPGGSLRLSCEASGFTFGDYAMHWVRQAPGKGLEWVSFISGDGAGRYYADSAKGRYTVARDNSKSTLSLEMNSLTPEDTAFYYCASYVRTVLPGGGYWYFDLWGRGTLVTVSS

SEQ ID NO: 170 - protein, 8 aa, synthetic construct
GFTFGDYA

SEQ ID NO: 171 - protein, 8 aa, synthetic construct
ISGDGAGR

SEQ ID NO: 172 - protein, 18 aa, synthetic construct
ASYVRTVLPGGGYWYFDL

SEQ ID NO: 173 - protein, 107 aa, synthetic construct
EIVLTQSPGTLSVSPGERVTLSCRASQSVGRYLAWYQQKTGQAPRLLVYDASNRATGIPARFSGSGSGTDFTLTISRLQPEDSAVYYCQQRSDWPPTFGGGTKVEIK

SEQ ID NO: 174 - protein, 6 aa, synthetic construct
QSVGRY

SEQ ID NO: 175 - skipped

SEQ ID NO: 176 - protein, 9 aa, synthetic construct
QQRSDWPPT

SEQ ID NO: 177 - protein, 123 aa, synthetic construct
EMRLLESGGGLVQPGGSLRVSCAASGFTFSSYSMSWVRQAPGKGLEWVSAISGSGGHSFFADSVKGRFSISRDNSKNMLYLQMNSLRAEDTAVYYCAKDDILMAALPNGFHVWGQGTLVIVSS

SEQ ID NO: 178 - protein, 8 aa, synthetic construct
GFTFSSYS

SEQ ID NO: 179 - protein, 8 aa, synthetic construct
ISGSGGHS

SEQ ID NO: 180 - protein, 16 aa, synthetic construct
AKDDILMAALPNGFHV

SEQ ID NO: 181 - protein, 108 aa, synthetic construct
SYVLTQSPSVPVAPGKTARITCGGDNIGSKSVQWYQQKPGQAPVVVVHDDNERPSGIPERFSGSNSGNTATLTISRVEAGDEADYYCQVWDRGSEHVVFGGGTKLTVL

SEQ ID NO: 182 - protein, 6 aa, synthetic construct
NIGSKS

SEQ ID NO: 183 - skipped

SEQ ID NO: 184 - protein, 11 aa, synthetic construct
QVWDRGSEHVV

SEQ ID NO: 185 - protein, 128 aa, synthetic construct
EVQLVASGGGLVRPGGSLRLSCAASGFMFRAHTMSWVRQAPGRGPEWISSISSGSSYIYSTDSLKGRFTISRDNARSSLFLHMNDLRTEDTAMYYCARDRGFHGSGVPSGYLEPFDLWGQGTMVTVSS

SEQ ID NO: 186 - protein, 8 aa, synthetic construct
GFMFRAHT

SEQ ID NO: 187 - protein, 8 aa, synthetic construct
ISSGSSYI

SEQ ID NO: 188 - protein, 21 aa, synthetic construct
ARDRGFHGSGVPSGYLEPFDL

SEQ ID NO: 189 - protein, 107 aa, synthetic construct
DIQMTQSPVSLSASVGDRVTITCRASQAISNSIAWYQQKPGKVPGLLVYAASRLENGVPSRFSGSGSGTDYTLTISSLQPEDFATYYCQQYFTVPRTFGQGTKVEVK

SEQ ID NO: 190 - protein, 6 aa, synthetic construct
QAISNS

SEQ ID NO: 191 - skipped

SEQ ID NO: 192 - protein, 9 aa, synthetic construct
QQYFTVPRT

SEQ ID NO: 193 - protein, 122 aa, synthetic construct
QVQLVQSGAEVKKPGASVKISCRPSGYIFNTHAIHWVRQAPGQRLEWMGWVNNRNGNTHYSQNFQGRVAINSDTSANTVYMTLSGLTFGDTAVYFCVREAYTGSFYDTFDVWGQGTTVTVSS

SEQ ID NO: 194 - protein, 8 aa, synthetic construct
GYIFNTHA

SEQ ID NO: 195 - protein, 8 aa, synthetic construct
VNNRNGNT

SEQ ID NO: 196 - protein, 15 aa, synthetic construct
VREAYTGSFYDTFDV

SEQ ID NO: 197 - protein, 108 aa, synthetic construct
DIQMTQSPSTLSAYVGDRVTITCRASQSVNGWLAWFHQQPGRAPKLLIYKASILEKGVPSRFSGSGSGTAFTLTISSLQPEDVGTYFCQQYNSYYSWTFGQGTKVEVK

SEQ ID NO: 198 - protein, 6 aa, synthetic construct
QSVNGW

SEQ ID NO: 199 - skipped

SEQ ID NO: 200 - protein, 10 aa, synthetic construct
QQYNSYYSWT

SEQ ID NO: 201 - protein, 117 aa, synthetic construct
KVQLVESGGALVKPGGSLRLSCTVSGYPFTTAWMSWVRQAPGKGLEWVGRIKNKVDGGTADYATPVKGRFTISRDDSRNILYLQMNSLKTEDTGVYYCATQHALDHWGQGTLVAVSP

SEQ ID NO: 202 - protein, 8 aa, synthetic construct
GYPFTTAW

SEQ ID NO: 203 - protein, 10 aa, synthetic construct
IKNKVDGGTA

SEQ ID NO: 204 - protein, 8 aa, synthetic construct
ATQHALDH

SEQ ID NO: 205 - protein, 107 aa, synthetic construct
SYVLTQPPSVSVAPGKTASITCGGEKIGDKNVHWYQQKPGQAPMVVIYYDSDRPSGIPERFSGSNSGNTATLTISRVEAGDEADYYCHVWDSSSNHKVFGGGTKLTV

SEQ ID NO: 206 - protein, 6 aa, synthetic construct
KIGDKN

SEQ ID NO: 207 - skipped

SEQ ID NO: 208 - protein, 11 aa, synthetic construct
HVWDSSSNHKV

SEQ ID NO: 209 - protein, 123 aa, synthetic construct
QVQLVESGGGVVQPGRSLRLTCAASQVTFRSYAMFWIRQAPGKGLEWVAMISNDGRYKYYADSVKGRFTISRDNSKSEFYLQMHSLRVEDTAVYFCAKGDTLFGVAQTGFDYWGQGTLVTVSS

SEQ ID NO: 210 - protein, 8 aa, synthetic construct
QVTFRSYA

SEQ ID NO: 211 - protein, 8 aa, synthetic construct
ISNDGRYK

SEQ ID NO: 212 - protein, 16 aa, synthetic construct
AKGDTLFGVAQTGFDY

SEQ ID NO: 213 - protein, 107 aa, synthetic construct
SYVLTQPPSVSVAPGKTASIACGGNNIGTKSVHWYQQKPGQAPVMVVYDDNERPSGIPERFSGSNSGNTATLTISRVEAGDEADYYCQVWDNSRDHLWVFGGGTKLT

SEQ ID NO: 214 - protein, 6 aa, synthetic construct
NIGTKS

SEQ ID NO: 215 - skipped

SEQ ID NO: 216 - protein, 12 aa, synthetic construct
QVWDNSRDHLWV

SEQ ID NO: 217 - protein, 122 aa, synthetic construct
EEQLVVSGGGLIQPGGSLKLSCTVSDFTFSRYELNWVRQTPGQRLEWLASTSTTGHNIHYAESVRGRFTISRDNGKNALSLQMNSLRADDTAAYYCARVRRVGGAHWFFDLWGRGALVTVSS

SEQ ID NO: 218 - protein, 8 aa, synthetic construct
DFTFSRYE

SEQ ID NO: 219 - protein, 8 aa, synthetic construct
TSTTGHNI

SEQ ID NO: 220 - protein, 15 aa, synthetic construct
ARVRRVGGAHWFFDL

SEQ ID NO: 221 - protein, 107 aa, synthetic construct
EIMMTQSPASLSVSPGERATLSCRASQSVARNLAWYQQKVGQAPRLLFYGASTRATGIPARFSGSGSGTDFTLSISSPQSEDVAVYYCQQYDDWPLTFGQGTRLEIK

SEQ ID NO: 222 - protein, 6 aa, synthetic construct
QSVARN

SEQ ID NO: 223 - skipped

SEQ ID NO: 224 - protein, 9 aa, synthetic construct
QQYDDWPLT

SEQ ID NO: 225 - protein, 118 aa, synthetic construct
QVQLQESGPGLVKPSETLSLTCSVSGGSIGKYFWTWIRQSPGKGLEWIGYIYYTGSTNYNPSLKSRVSMSVDSSRNEFSLKLSSVTATDTAVYYCARPYGDYDAFDIWGQGTMVTVSS

SEQ ID NO: 226 - protein, 8 aa, synthetic construct
GGSIGKYF

SEQ ID NO: 227 - protein, 7 aa, synthetic construct
IYYTGST

SEQ ID NO: 228 - protein, 12 aa, synthetic construct
ARPYGDYDAFDI

SEQ ID NO: 229 - protein, 110 aa, synthetic construct
QSVLTQPPSVSGTPGQRVTISCSGSRSNIGGNTVHWYQQFPGMAPKVLLYSNNERPSGVPDRFSGSKSGTSASLAISGLRSEDEANYYCAAWDDSLKGVVFGGGTKLTVL

SEQ ID NO: 230 - protein, 8 aa, synthetic construct
RSNIGGNT

SEQ ID NO: 231 - skipped

SEQ ID NO: 232 - protein, 11 aa, synthetic construct
AAWDDSLKGVV

SEQ ID NO: 233 - protein, 122 aa, synthetic construct
QVQLVESGGGVVRPGRSLRLSCVASGFTFSNYGMHWVRQAPGKGLQWVAGLWSDGSQKFYADSVKGRFTISRDNSKNTLYLQMNNLRAEDTAVYFCPRDGSGNNPSSFFDSWGQGILVTVSS

SEQ ID NO: 234 - protein, 8 aa, synthetic construct
GFTFSNYG

SEQ ID NO: 235 - protein, 8 aa, synthetic construct
LWSDGSQK

SEQ ID NO: 236 - protein, 15 aa, synthetic construct
PRDGSGNNPSSFFDS

SEQ ID NO: 237 - protein, 108 aa, synthetic construct
EIVLTQSPGTLSLSPGERATLSCRASLTVAGIYLTWYQQKRGQAPRLLIYGASNRAAGIPDRFSGSGSGTAFTLTISRLKPEDFAVYYCQVYGNSRWTFGQGTKVEVK

SEQ ID NO: 238 - protein, 7 aa, synthetic construct
LTVAGIY

SEQ ID NO: 239 - skipped

SEQ ID NO: 240 - protein, 9 aa, synthetic construct
QVYGNSRWT

SEQ ID NO: 241 - protein, 125 aa, synthetic construct
QVQVVQSGGGVVQPGDSLRLSCAASGFALSSFGMQWVRQAPGKGLEWVAVIWFDGSNKFYADSVKGRFTISRDSSKNTVFLQMNSLRTNDTAIYYCARGYGDVFSGYSPNYFDYWGQGSRVTVAS

SEQ ID NO: 242 - protein, 8 aa, synthetic construct
GFALSSFG

SEQ ID NO: 243 - protein, 8 aa, synthetic construct
IWFDGSNK

SEQ ID NO: 244 - protein, 18 aa, synthetic construct
ARGYGDVFSGYSPNYFDY

SEQ ID NO: 245 - protein, 110 aa, synthetic construct
QSVLTQPPSVSGAPGQRVTISCTGSSSNIGARCDVHWYQQLPGAAPKLLIYSNTNRPSGVPARFSASKSGTSASLAITGLRAEDEADYYCQSCDSSLSGYVFGTGTKVTV

SEQ ID NO: 246 - protein, 9 aa, synthetic construct
SSNIGARCD

SEQ ID NO: 247 - skipped

SEQ ID NO: 248 - protein, 11 aa, synthetic construct
QSCDSSLSGYV

SEQ ID NO: 249 - protein, 123 aa, synthetic construct
QVQFVQSGAEVKKPGASVKVSCRTSGYTFTRYAMHWVRQAPGQRLEWMGWINAGNGLTKYSQKFQGRVTITRDTSANILYMELSSLRSEDTAVYYCARVGLSDTGDPAPFDYWGQGTLVTVSS

SEQ ID NO: 250 - protein, 8 aa, synthetic construct
GYTFTRYA

SEQ ID NO: 251 - protein, 8 aa, synthetic construct
INAGNGLT

SEQ ID NO: 252 - protein, 16 aa, synthetic construct
ARVGLSDTGDPAPFDY

SEQ ID NO: 253 - protein, 111 aa, synthetic construct
QSVLTQPPSVTGAPGQRVTISCTGRSSNIGAGYDLHWYQQLPGTAPKLLIYGNGHRPSGVPDRFSGSKSGTSASLVITGLQAEDEADYYCHSYDRSLSEVVFGGGTKLTVL

SEQ ID NO: 254 - protein, 9 aa, synthetic construct
SSNIGAGYD

SEQ ID NO: 255 - skipped

SEQ ID NO: 256 - protein, 11 aa, synthetic construct
HSYDRSLSEVV

SEQ ID NO: 257 - protein, 125 aa, synthetic construct
EIQMVQSGAVVKKPGESLKISCQGSGYSFSDFWIGWVRQMPGKGLEWMGIIHPEDSYTQYSPSFRGQVTISADKSIRTAYLQWSSLQASDTAIYYCAKRGGGVVNSYYYYAMDVWGQGTSVTVSS

SEQ ID NO: 258 - protein, 8 aa, synthetic construct
GYSFSDFW

SEQ ID NO: 259 - protein, 8 aa, synthetic construct
IHPEDSYT

SEQ ID NO: 260 - protein, 18 aa, synthetic construct
AKRGGGVVNSYYYYAMDV

SEQ ID NO: 261 - protein, 107 aa, synthetic construct
DIQMTQSPSSVSASVGDRVTIACRASQGIGGWLAWYQQKPGKAPRLLIYAASTLQSGVPSRFSGSGSGTYFTLAISSLQPEDFATYYCQQTNSFPYTFGQGTKVEIK

SEQ ID NO: 262 - protein, 6 aa, synthetic construct
QGIGGW

SEQ ID NO: 263 - skipped

SEQ ID NO: 264 - protein, 9 aa, synthetic construct
QQTNSFPYT

SEQ ID NO: 265 - protein, 124 aa, synthetic construct
QVQLVQSGAEVKKPGASVRVSCKASGYTFSTHNMHWVRQAPGQGLEWMGRINADTGNSKYSQKFLGRVTINRDTSANTVYMELRGLRPEDTAVYYCARELEGADTGWDSWFDPWGQGTLVTVSS

SEQ ID NO: 266 - protein, 8 aa, synthetic construct
GYTFSTHN

SEQ ID NO: 267 - protein, 8 aa, synthetic construct
INADTGNS

SEQ ID NO: 268 - protein, 17 aa, synthetic construct
ARELEGADTGWDSWFDP

SEQ ID NO: 269 - protein, 107 aa, synthetic construct
SNELTQPPSVSVSPGQTASIPCSGDKLGDKYASWYQQKPGRSPVVVIYQDTKRPSGIPERFSGSNSGNTATLTISGTQAMDEAAYYCQAWDSSTAAVFGGGTKLTVL

SEQ ID NO: 270 - protein, 6 aa, synthetic construct
KLGDKY

SEQ ID NO: 271 - skipped

SEQ ID NO: 272 - protein, 10 aa, synthetic construct
QAWDSSTAAV

SEQ ID NO: 273 - protein, 118 aa, synthetic construct
EVQLVESEGGVVRPGGSLRLSCAASGFTFDNYGMSWVRQAPGKGLEWVSRINWNGGGTDYADSVKGRFTISRDNARNSLYLQMNSLRVEDTAFYYCVRDEDWNQFDPWGQGTLVTVSS

SEQ ID NO: 274 - protein, 8 aa, synthetic construct
GFTFDNYG

SEQ ID NO: 275 - protein, 8 aa, synthetic construct
INWNGGGT

SEQ ID NO: 276 - protein, 11 aa, synthetic construct
VRDEDWNQFDP

SEQ ID NO: 277 - protein, 110 aa, synthetic construct
HSALTQPASVSGSLGQSITISCTGTSSDVGGYNFVSWYQQHPGKAPKLIIYDVSSRPSGVSNRFSGSKSGKTASLTISGLQTEDEADYHCSSYSRSSTVVFGGGTKVTVL

SEQ ID NO: 278 - protein, 9 aa, synthetic construct
SSDVGGYNF

SEQ ID NO: 279 - skipped

SEQ ID NO: 280 - protein, 10 aa, synthetic construct
SSYSRSSTVV

SEQ ID NO: 281 - protein, 124 aa, synthetic construct
QVQLVESGGGVVQPGRSLRLSCAASGFSFSDYGLHWVRQAPGKGLEWVAGILSDGSQTFYADSVRGRLTISRDNSKNTLFLQMNSLRAADTAVYYCSRDRVSSSGWYVWDFGLWGRGTLVTVSS

SEQ ID NO: 282 - protein, 8 aa, synthetic construct
GFSFSDYG

SEQ ID NO: 283 - protein, 8 aa, synthetic construct
ILSDGSQT

SEQ ID NO: 284 - protein, 17 aa, synthetic construct
SRDRVSSSGWYVWDFGL

SEQ ID NO: 285 - protein, 107 aa, synthetic construct
EIVMTQSPATLSVSPGERATLSCRASQSVSTNLAWYQQKPGQAPILLIYDASARATGVPDRFSGSGSRREFTLTISSLQSEDSAVYHCQQHHNWPITFGQGTRLEIR

SEQ ID NO: 286 - protein, 6 aa, synthetic construct
QSVSTN

SEQ ID NO: 287 - skipped

SEQ ID NO: 288 - protein, 9 aa, synthetic construct
QQHHNWPIT

SEQ ID NO: 289 - protein, 123 aa, synthetic construct
EVQLVESGGGLVQPSGSLRLSCTASGFIFSNYEMNWVRQAPGKGLEWVSYISHGGSTIYYADSVKGRFTISRDNAKNSLYLQMNSLRAEDTAVYYCARDRAGRDYVFDAFDSWGQGTMVTVSS

SEQ ID NO: 290 - protein, 8 aa, synthetic construct
GFIFSNYE

SEQ ID NO: 291 - protein, 8 aa, synthetic construct
ISHGGSTI

SEQ ID NO: 292 - protein, 16 aa, synthetic construct
ARDRAGRDYVFDAFDS

SEQ ID NO: 293 - protein, 106 aa, synthetic construct
SIELTQPPSVSVSPGQTASITCSGDKLGDKYACWYQQKPGQSPVLVIYQDDKRPSGIPERFSASNSGNTATLTISGTQAMDEADYYCQAWDSTNWVFGGGTKLTVL

SEQ ID NO: 294 - protein, 6 aa, synthetic construct
KLGDKY

SEQ ID NO: 295 - skipped

SEQ ID NO: 296 - protein, 9 aa, synthetic construct
QAWDSTNWV

SEQ ID NO: 297 - protein, 124 aa, synthetic construct
QVQLVQSGAEVKKPGASVKVSCKASGYTFTNYAMHWVRQAPGQRLEWMGWINADNGNTKYSQKFQGRVTITRDTSASTVYMQLSSLRSDDTAVYYCARVLEGADTGWDNWFDPWGQGTLVTVSS

SEQ ID NO: 298 - protein, 8 aa, synthetic construct
GYTFTNYA

SEQ ID NO: 299 - protein, 8 aa, synthetic construct
INADNGNT

SEQ ID NO: 300 - protein, 17 aa, synthetic construct
ARVLEGADTGWDNWFDP

SEQ ID NO: 301 - protein, 107 aa, synthetic construct; identical to SEQ ID NO: 269

SEQ ID NO: 302 - protein, 6 aa, synthetic construct
KLGDKY

SEQ ID NO: 303 - skipped

SEQ ID NO: 304 - protein, 10 aa, synthetic construct
QAWDSSTAAV

SEQ ID NO: 305 - protein, 123 aa, synthetic construct
QVQLVQSGAEVKKPGASVKVSCKASGYTFTWYAMHWVRQAPGQRLEWRGWGSAGNGITKDSQKFQGRVTITRDTSASTAYMELSSLRSEDTAVYYCARVGLSDTGDPAPFDYWGQGTLVTVSS

SEQ ID NO: 306 - protein, 8 aa, synthetic construct
GYTFTWYA

SEQ ID NO: 307 - protein, 8 aa, synthetic construct
GSAGNGIT

SEQ ID NO: 308 - protein, 16 aa, synthetic construct
ARVGLSDTGDPAPFDY

SEQ ID NO: 309 - protein, 111 aa, synthetic construct
QSVLTQPPSVSGAPGQRVTISCTGSSSNIGAGFDVHWYQQLPGTAPKVLIYSTNNRPSGVPDRFSGSKSATSASLAITGLQAEDEADYYCQSYDSSLSGVVFGGGTKLTVL

SEQ ID NO: 310 - protein, 9 aa, synthetic construct
SSNIGAGFD

SEQ ID NO: 311 - skipped

SEQ ID NO: 312 - protein, 11 aa, synthetic construct
QSYDSSLSGVV

SEQ ID NO: 313 - protein, 120 aa, synthetic construct
QVQLVEYGGGVVQPGRSLRLSCAASGFTFSTYGIHWVRQAPGKGLEWVALIWKDGTNKYYADSVKGRFTISRDNSKNTVYLQMNGLRAEDTAVYYCAREALVLVTAYDLWGQGTLVAVSS

SEQ ID NO: 314 - protein, 8 aa, synthetic construct
GFTFSTYG

SEQ ID NO: 315 - protein, 8 aa, synthetic construct
IWKDGTNK

SEQ ID NO: 316 - protein, 13 aa, synthetic construct
AREALVLVTAYDL

SEQ ID NO: 317 - protein, 109 aa, synthetic construct
DIQLTQSPSSLSAFVGDRVTITCRASQSVRDYLNWYQHKPGKAPKLLIYGASALQSGVPSRFSGSGSGTDFTLTISSLQPEDLATYYCQQSYSTPESFTFGPGTKIHIK

SEQ ID NO: 318 - protein, 6 aa, synthetic construct
QSVRDY

SEQ ID NO: 319 - skipped

SEQ ID NO: 320 - protein, 11 aa, synthetic construct
QQSYSTPESFT

SEQ ID NO: 321 - protein, 129 aa, synthetic construct
QLQLQESGPGLVKPSETLTLTCTVSGGSIRSSFYWGWIRQPPGKGLEWIGSIYWSGSTYYNPSLKSRVSVSVDTSKNQFSLKLSSVTAADTAVYFCARQAYVKSHGWAAIPSYYYIDVWGKGTTVTVSS

SEQ ID NO: 322 - protein, 9 aa, synthetic construct
GGSIRSSFY

SEQ ID NO: 323 - protein, 7 aa, synthetic construct
IYWSGST

SEQ ID NO: 324 - protein, 22 aa, synthetic construct
ARQAYVKSHGWAAIPSYYYIDV

SEQ ID NO: 325 - protein, 111 aa, synthetic construct
QSVLTQPPSVSGAPGQRVTISCTGSSSNIGAAYDVHWYQQLPGVAPKLLIFANSNRPSGVPDRFSGSKSGTSASLAITGLQAEDEADYYCQSYDSSLSGWVFGEGTKLTVL

SEQ ID NO: 326 - protein, 9 aa, synthetic construct
SSNIGAAYD

SEQ ID NO: 327 - skipped

SEQ ID NO: 328 - protein, 11 aa, synthetic construct
QSYDSSLSGWV

SEQ ID NO: 329 - protein, 118 aa, synthetic construct
QVQLVESGGGVVQPGRSLRLSCAASGFTFSNYPMHWVRQAPGKGLEWVSLISYDGSYQYYPDSLKGRFTISRDNSKDTLYLQMNSLRFDDTAVYYCARASFANHLDYWGQGALLTVSS

SEQ ID NO: 330 - protein, 8 aa, synthetic construct
GFTFSNYP

SEQ ID NO: 331 - protein, 8 aa, synthetic construct
ISYDGSYQ

SEQ ID NO: 332 - protein, 11 aa, synthetic construct
ARASFANHLDY

SEQ ID NO: 333 - protein, 108 aa, synthetic construct
EIVLTQSPGTLSLVPGARATLSCRASQSITSDYLAWYQQRPGQAPRLLIYGASSRATGIPDRFSGSGSGTDFTLTISRLEPQDFAVYYCHQYGNLPRTFGQGTKLEIK

SEQ ID NO: 334 - protein, 7 aa, synthetic construct
QSITSDY

SEQ ID NO: 335 - skipped

SEQ ID NO: 336 - protein, 9 aa, synthetic construct
HQYGNLPRT

SEQ ID NO: 337 - protein, 118 aa, synthetic construct
QVQLVESGGGVVQPGRSLRLSCAASGFTFSSFPMAWVRQAPGKGLEWVTLISYDGTYKYYADYVKGRFAISRDNSKDTLFLQMNSLRPEDTAVYYCAREHFGSAFDSWGQGTLVTVSS

SEQ ID NO: 338 - protein, 8 aa, synthetic construct
GFTFSSFP

SEQ ID NO: 339 - protein, 8 aa, synthetic construct
ISYDGTYK

SEQ ID NO: 340 - protein, 11 aa, synthetic construct
AREHFGSAFDS

SEQ ID NO: 341 - protein, 107 aa, synthetic construct
EIVLTQSPATLSLSPGERATLSCRASQTISSYLAWYQQKPGQSPRLLIYDVSTRATGIPARFSGSGSGTDFTLTISSLETEDFAVYYCQQRSNWPRTFGQGTKLEIR

SEQ ID NO: 342 - protein, 6 aa, synthetic construct
QTISSY

SEQ ID NO: 343 - skipped

SEQ ID NO: 344 - protein, 9 aa, synthetic construct
QQRSNWPRT

SEQ ID NO: 345 - protein, 117 aa, synthetic construct
QVQLVQSGAEVKKPGSSVKVSCKASGGGFNRDAVSWVRQAPGQGLEWMGRIIPLLRIGNNAQKFQDRVTITADKFTNTVYLQVSGLRSEDTAVYYCAREKGDALDLWGQGTLVTVSF

SEQ ID NO: 346 - protein, 8 aa, synthetic construct
GGGFNRDA

SEQ ID NO: 347 - protein, 8 aa, synthetic construct
IIPLLRIG

SEQ ID NO: 348 - protein, 10 aa, synthetic construct
AREKGDALDL

SEQ ID NO: 349 - protein, 108 aa, synthetic construct
EIVLTQSPGTLSLSPGERATLSCGASQTVSSSYLAWYQQKPGQAPRLLIYASSSRATGIPERFSGSGSGTDFTLTINRLEPEDFAVYYCQQYVTSPYTFGQGTKLEIK

SEQ ID NO: 350 - protein, 7 aa, synthetic construct
QTVSSSY

SEQ ID NO: 351 - skipped

SEQ ID NO: 352 - protein, 9 aa, synthetic construct
QQYVTSPYT

SEQ ID NO: 353 - protein, 123 aa, synthetic construct
QVQLVQSGPEVKKPGASVKVSCKASGYSFSSYGISWVRQAPGQGLEWMGWISTLNGNTNYAQNFQGRVTVTTDTSSTTVYMELTRLTSDDTAVYYCARDGRRYTSGWYYFANWGQGTLVIVSS

SEQ ID NO: 354 - protein, 8 aa, synthetic construct
GYSFSSYG

SEQ ID NO: 355 - protein, 8 aa, synthetic construct
ISTLNGNT

SEQ ID NO: 356 - protein, 16 aa, synthetic construct
ARDGRRYTSGWYYFAN

SEQ ID NO: 357 - protein, 108 aa, synthetic construct
DIVLTQSPGSLSVSPGERVTLSCRARQGVNSNLAWYQQKPGQAPRLLIYDASTRATGIPARFSGSGSGTEFTLTISSLQSEDFAVYYCQQYKTWPPVTFGGGTKVQIK

SEQ ID NO: 358 - protein, 6 aa, synthetic construct
QGVNSN

SEQ ID NO: 359 - skipped

SEQ ID NO: 360 - protein, 10 aa, synthetic construct
QQYKTWPPVT

SEQ ID NO: 361 - protein, 122 aa, synthetic construct
QVQLMQSGAEVKKPGSSVKVSCKASGGNFRSYGFSWVRQAPGQGLEWMGRIIPIFGVTNYAQKFRDRVTITADKSTSTAYMDLRSLRSEDTAVYYCARSPTVTNNFWYFDLWGRGTLVTVSS

SEQ ID NO: 362 - protein, 8 aa, synthetic construct
GGNFRSYG

SEQ ID NO: 363 - protein, 8 aa, synthetic construct
IIPIFGVT

SEQ ID NO: 364 - protein, 15 aa, synthetic construct
ARSPTVTNNFWYFDL

SEQ ID NO: 365 - protein, 108 aa, synthetic construct
VIQMTQSPSSLAASVGGSVTITCRASQAISNSVAWYQQKPGEAPKLLLFEASRLASGVPSRFSGSGSGTDYTLTISSLQPEDFATYYCQHYYNILPFTFGPGTKVDIK

SEQ ID NO: 366 - protein, 6 aa, synthetic construct
QAISNS

SEQ ID NO: 367 - skipped

SEQ ID NO: 368 - protein, 10 aa, synthetic construct
QHYYNILPFT

SEQ ID NO: 369 - protein, 119 aa, synthetic construct
QVQLVQSGAEVKKPGSSMKVSCKASGGTFSNYAVSWVRQAPGQGLEWMGKIIPVFGATQYTQKFQGRITMTADRSTGTAFLELSGLTSEDTAIYYCARHWARGRWFDYWGQGTLVTVSS

SEQ ID NO: 370 - protein, 8 aa, synthetic construct
GGTFSNYA

SEQ ID NO: 371 - protein, 8 aa, synthetic construct
IIPVFGAT

SEQ ID NO: 372 - protein, 12 aa, synthetic construct
ARHWARGRWFDY

SEQ ID NO: 373 - protein, 107 aa, synthetic construct
DIQVTQSPSSLSASVGDRVTITCQATLDTGNSLNWYQQRPGKAPQLLIYDTSNLATGVPSRFSGSGSETQFTLTINNVQPEDFATYYCQQFDNLLFTFGGGTKVDMK

SEQ ID NO: 374 - protein, 6 aa, synthetic construct
LDTGNS

SEQ ID NO: 375 - skipped

SEQ ID NO: 376 - protein, 9 aa, synthetic construct
QQFDNLLFT

SEQ ID NO: 377 - protein, 117 aa, synthetic construct
QVQLLQSGAEVKKPGSSVKVSCKASGGSFNRDAISWVRQAPGQGLEWMGRIIPILKIGNNAQKLQGRVTITADKFTGTVYMELSSLRSDDTAMYYCTREKGDAFDIWGQGTMVTVSS

SEQ ID NO: 378 - protein, 8 aa, synthetic construct
GGSFNRDA

SEQ ID NO: 379 - protein, 8 aa, synthetic construct
IIPILKIG

SEQ ID NO: 380 - protein, 10 aa, synthetic construct
TREKGDAFDI

SEQ ID NO: 381 - protein, 108 aa, synthetic construct
EIVLTQSPGTLSLSPGERATLSCRASQSVSSSYLAWYQQKPGQTPRLLIYATSSRATGIPDRFSGSGSGTDFTLTISRLQPEDFAVYYCQQYGSSPYTFGQGTKLEIK

SEQ ID NO: 382 - protein, 7 aa, synthetic construct
QSVSSSY

SEQ ID NO: 383 - skipped

SEQ ID NO: 384 - protein, 9 aa, synthetic construct
QQYGSSPYT

SEQ ID NO: 385 - protein, 119 aa, synthetic construct
QVQLVQSGAEVKKPGSSVKVSCKASGGSFRSDAMNWVRQAPGQGLEWLGKIIPMLRIANYAQRLQGRVSITVDRSRTTVYMELSSLRSEDTAVYYCARNDDTDMSLDSWGQGTLVTVSS

SEQ ID NO: 386 - protein, 8 aa, synthetic construct
GGSFRSDA

SEQ ID NO: 387 - protein, 8 aa, synthetic construct
IIPMLRIA

SEQ ID NO: 388 - protein, 12 aa, synthetic construct
ARNDDTDMSLDS

SEQ ID NO: 389 - protein, 109 aa, synthetic construct
QSALTQPPSASGSPGQSVTISCTGTSSDIGAYDFVAWYQHHPGKAPKLMIYKVNQRPSGVPARFYGSKSGNTASLTVSGLQADDEADYYCSSYAGSNSLVFGGGTKLTV

SEQ ID NO: 390 - protein, 9 aa, synthetic construct
SSDIGAYDF

SEQ ID NO: 391 - skipped

SEQ ID NO: 392 - protein, 10 aa, synthetic construct
SSYAGSNSLV

SEQ ID NO: 393 - protein, 119 aa, synthetic construct
QVQLVQSGAEVKKPGSSVKVSCKASGGTFRNDAVSWVRQAPGQGLEWMGRIIPVFGTTTYTQKFQGRVTMTADRSTGTAFLELSSLTSEDTAIYYCARHRARGRWFDYWGQGTLVTVSS

SEQ ID NO: 394 - protein, 8 aa, synthetic construct
GGTFRNDA

SEQ ID NO: 395 - protein, 8 aa, synthetic construct
IIPVFGTT

SEQ ID NO: 396 - protein, 12 aa, synthetic construct
ARHRARGRWFDY

SEQ ID NO: 397 - protein, 114 aa, synthetic construct
DIVLTQSPDSLAVSLGERATINCKSSQSVLYSSNNKNYLAWYQQKPGQPPKLLIYWASTRESGVPDRFSGSGSGTDFTLTISSLQAEDVAVYYCQQYYDLRSITFGQGTRLEIK

SEQ ID NO: 398 - protein, 12 aa, synthetic construct
QSVLYSSNNKNY

SEQ ID NO: 399 - skipped

SEQ ID NO: 400 - protein, 10 aa, synthetic construct
QQYYDLRSIT

SEQ ID NO: 401 - protein, 119 aa, synthetic construct
QVHLVQSGAEVKRPGSSVKVSCKPSGETFRNYAINWLRQAPGQGLEWMGSIIPIIGITNYAQRFKGRVTISADRSTGTAYMELSSLRSDDTATFYCARGFSGYNYFDMWGQGTRVTVSS

SEQ ID NO: 402 - protein, 8 aa, synthetic construct
GETFRNYA

SEQ ID NO: 403 - protein, 8 aa, synthetic construct
IIPIIGIT

SEQ ID NO: 404 - protein, 12 aa, synthetic construct
ARGFSGYNYFDM

SEQ ID NO: 405 - protein, 110 aa, synthetic construct
QSVLTQPPSVSAAPGQRVTISCSGSTSNIGNNYVSWYKQVPETAPKVLIYNNDQRPSEIPDRISGSKSGTSATLGITGLQTGDEADYYCGSWDSSLSAVVFGGGTKLTVL

SEQ ID NO: 406 - protein, 8 aa, synthetic construct
TSNIGNNY

SEQ ID NO: 407 - skipped

SEQ ID NO: 408 - protein, 11 aa, synthetic construct
GSWDSSLSAVV

SEQ ID NO: 409 - protein, 123 aa, synthetic construct
QLQLQESGPGLVKPSETLSLTCTVSGGSISSYPYYWGWIRQPPGKGLEWIGTIYYSGKTYYTPSLRSRVTISVDTSKNQFSLKLKSVTAADTAVYFCARQEGFGTSWYHFDYWGPGTLVAVSS

SEQ ID NO: 410 - protein, 10 aa, synthetic construct
GGSISSYPYY

SEQ ID NO: 411 - protein, 7 aa, synthetic construct
IYYSGKT

SEQ ID NO: 412 - protein, 15 aa, synthetic construct
ARQEGFGTSWYHFDY

SEQ ID NO: 413 - protein, 113 aa, synthetic construct
DIVMTQSPDSLAVSLGERATINCKSSQSLLYSSNNQNYLAWYQLKPGQPPKVVIYWASTRESGVPDRFSGSGSGTDFTLTISSLQAEDLAVYYCQQYYNTPLTFGQGTRLEIK

SEQ ID NO: 414 - protein, 12 aa, synthetic construct
QSLLYSSNNQNY

SEQ ID NO: 415 - skipped

SEQ ID NO: 416 - protein, 9 aa, synthetic construct
QQYYNTPLT

SEQ ID NO: 417 - protein, 116 aa, synthetic construct
QVQLLQSGTEVKKPGSSVRVSCKASGGIIGRDAINWVRQAPGQRLEWMGRIIPLIGVTNYAPKFQDRVTISADKFTNAVYMQLSRLTSDDTAVYFCARDPGYGDSWGQGTLISVSS

SEQ ID NO: 418 - protein, 8 aa, synthetic construct
GGIIGRDA

SEQ ID NO: 419 - protein, 8 aa, synthetic construct
IIPLIGVT

SEQ ID NO: 420 - protein, 9 aa, synthetic construct
ARDPGYGDS

SEQ ID NO: 421 - protein, 108 aa, synthetic construct
EIVLTQSPGTLSLSPGERATLSCRASQSVSRSYFAWFQQKPGQAPRLLIYGTSSRATGIPDRFSGSGSGTDFTLTISRLEPEDFAVYYCLQYVTSPWTFGQGTKVEIR

SEQ ID NO: 422 - protein, 7 aa, synthetic construct
QSVSRSY

SEQ ID NO: 423 - skipped

SEQ ID NO: 424 - protein, 9 aa, synthetic construct
LQYVTSPWT

SEQ ID NO: 425 - protein, 119 aa, synthetic construct
QVQLVQSGAEVKKPGSSVKVSCKASGGTFSREAINWVRQAPGQGLQWIGRIIPVIGILNYAQKFQGRVTITADKYTNTAYLSLSNLRFEDTAIYFCARQGDYSMYLEDWGQGTLVTVSS

SEQ ID NO: 426 - protein, 8 aa, synthetic construct
GGTFSREA

SEQ ID NO: 427 - protein, 8 aa, synthetic construct
IIPVIGIL

SEQ ID NO: 428 - protein, 12 aa, synthetic construct
ARQGDYSMYLED

SEQ ID NO: 429 - protein, 110 aa, synthetic construct
QSVLTQPPSVSAAPGQKVTISCSGSSSNIGNNHVCWYQQFPGTAPKLLIYDNNKRPSGIPDRFSGSKSGTSATLGITGLQTGDEADYYCGTWDSSLSAGVFGGGTKLTVL

SEQ ID NO: 430 - protein, 8 aa, synthetic construct
SSNIGNNH

SEQ ID NO: 431 - skipped

SEQ ID NO: 432 - protein, 11 aa, synthetic construct
GTWDSSLSAGV

SEQ ID NO: 433 - protein, 124 aa, synthetic construct
QVQLVESGGGVVQPGRSLRLSCAASGFRFSYYGLNWIRQAPGKGLEWMAVISYDGRHKSYVDSVKGRFTIARDNSKNTLYLQMDSLSAEDTAVYYCAKSSVLYSTQDGGAFDYWGQGTVVTVSS

SEQ ID NO: 434 - protein, 8 aa, synthetic construct
GFRFSYYG

SEQ ID NO: 435 - protein, 8 aa, synthetic construct
ISYDGRHK

SEQ ID NO: 436 - protein, 17 aa, synthetic construct
AKSSVLYSTQDGGAFDY

SEQ ID NO: 437 - protein, 109 aa, synthetic construct
SYVLTQPPSVSLAPGKTARITCGGTDIGSKSVHWYQQKPGQAPVLVVYDDIDRPSGIPERFSGSNSGNTATLTISRVEAGDEADYYCQVWDSSSDHFYVFGTGTKVTVL

SEQ ID NO: 438 - protein, 6 aa, synthetic construct
DIGSKS

SEQ ID NO: 439 - skipped

SEQ ID NO: 440 - protein, 12 aa, synthetic construct
QVWDSSSDHFYV

SEQ ID NO: 441 - protein, 130 aa, synthetic construct
QVQLQESGPGLVRPSQTLSLTCTVSGGSINTGDSHWSWIRQTPGKGLEWIGNIFYSGNTHYNPSLKSRLSLSLDTSKNQFFLKLRSVTAADTAVYYCARFDCSGNSCYSPRAYYYGMDVWGRGTTVTVSS

SEQ ID NO: 442 - protein, 10 aa, synthetic construct
GGSINTGDSH

SEQ ID NO: 443 - protein, 7 aa, synthetic construct
IFYSGNT

SEQ ID NO: 444 - protein, 22 aa, synthetic construct
ARFDCSGNSCYSPRAYYYGMDV

SEQ ID NO: 445 - protein, 113 aa, synthetic construct
DIVMTQSPLSLAVTPGEPASISCRSSQSLLHSNGYNYLDWYLQKPGQSPQLLIYLGSNRALGVPDRFSGSGSGTDFTLKISRVEAEDVGVYYCMQALQARPITFGPGTKVHIK

SEQ ID NO: 446 - protein, 11 aa, synthetic construct
QSLLHSNGYNY

SEQ ID NO: 447 - skipped

SEQ ID NO: 448 - protein, 10 aa, synthetic construct
MQALQARPIT

SEQ ID NO: 449 - protein, 118 aa, synthetic construct
QVQLVESGGGVVHPGRSLRLSCAASGFAFTSYPMHWVRQAPGKGLEWVALIPYDATNTYYADSVTGRFTISRDNSNNILFLQMNSLRVEDTAVYYCTRGNVGHRFDPWGLGTLVIVSP

SEQ ID NO: 450 - protein, 8 aa, synthetic construct
GFAFTSYP

SEQ ID NO: 451 - protein, 8 aa, synthetic construct
IPYDATNT

SEQ ID NO: 452 - protein, 11 aa, synthetic construct
TRGNVGHRFDP

SEQ ID NO: 453 - protein, 113 aa, synthetic construct
DIVMTQSPDSLAVSLGERATINCKSSQNVLYSFNNKNYLAWFQQKPGQPPKLLIYWASTREFGVPDRFSGSGSGTDFTLTISSLQAEDVAVYYCQQYYSTPLTFGGGTKVEIK

SEQ ID NO: 454 - protein, 12 aa, synthetic construct
QNVLYSFNNKNY

SEQ ID NO: 455 - skipped

SEQ ID NO: 456 - protein, 9 aa, synthetic construct
QQYYSTPLT

SEQ ID NO: 457 - protein, 123 aa, synthetic construct
EVKLLESGGALVRPGGSLRLSCAASGFTFTSYAMSWVRQAPGKGLEWVSFIYSGASGTFYANSVKGRFTISRDNSKNTVYLQMNSLRAEDTAIYYCAKGGRWNGDADDAFHTWGQGTMVTVSS

SEQ ID NO: 458 - protein, 8 aa, synthetic construct
GFTFTSYA

SEQ ID NO: 459 - protein, 8 aa, synthetic construct
IYSGASGT

SEQ ID NO: 460 - protein, 16 aa, synthetic construct
AKGGRWNGDADDAFHT

SEQ ID NO: 461 - protein, 110 aa, synthetic construct
QSVLTQPPSASGTPGQRVTISCSGSSSNIGSNTVNWYQQLPGTAPKLLIYSNNQRPSGVPDRFSGSKSGTSASLAISGLQSEDEADYYCAAWDDSLNGVVFGGGTKLTVL

SEQ ID NO: 462 - protein, 8 aa, synthetic construct
SSNIGSNT

SEQ ID NO: 463 - skipped

SEQ ID NO: 464 - protein, 11 aa, synthetic construct
AAWDDSLNGVV

SEQ ID NO: 465 - protein, 121 aa, synthetic construct
EVQLVESGGGLVQPGGSLRLSCAGSGFRFSNFEMNWVRQAPGKGLEWISYIGPRGTNIYYASSVWDRFTISRDDARNSVYLQMSSLRAEDTAVYYCATTHKSGWTKLFDDWGQGTLVTVSS

SEQ ID NO: 466 - protein, 8 aa, synthetic construct
GFRFSNFE

SEQ ID NO: 467 - protein, 8 aa, synthetic construct
IGPRGTNI

SEQ ID NO: 468 - protein, 14 aa, synthetic construct
ATTHKSGWTKLFDD

SEQ ID NO: 469 - protein, 107 aa, synthetic construct
DIQMTQSPSSVSASVGDRVTITCRASQNINSWLAWYQQKPGQAPKILIYATSRLESGVPSRFSGSRYGTDFTLTINSLQPEDSATYYCQQANSFPITFGPGTRLEIK

SEQ ID NO: 470 - protein, 6 aa, synthetic construct
QNINSW

SEQ ID NO: 471 - skipped

SEQ ID NO: 472 - protein, 9 aa, synthetic construct
QQANSFPIT

SEQ ID NO: 473 - protein, 120 aa, synthetic construct
EVQLVESGGGVVQPGRSLRLSCAASGFTFEHYAMHWVRQAPGKGLERVAGISWIGDNIVYADSVKGRFTISRDNAKNSLTLQMNSLRPEDTALYYCVKAFDILTGLFDHWGHGTLVTVSS

SEQ ID NO: 474 - protein, 8 aa, synthetic construct
GFTFEHYA

SEQ ID NO: 475 - protein, 8 aa, synthetic construct
ISWIGDNI

SEQ ID NO: 476 - protein, 13 aa, synthetic construct
VKAFDILTGLFDH

SEQ ID NO: 477 - protein, 108 aa, synthetic construct
EIVMTQSPATLSVSPGERATLSCRASQTITRNLAWYQHKPGQAPRLLMYGASIRATGVPDRFSGSGSGTEFTLTISSLRSEDFAVYYCQQYNQWPRYTFGQGTKLEIK

SEQ ID NO: 478 - protein, 6 aa, synthetic construct
QTITRN

SEQ ID NO: 479 - skipped

SEQ ID NO: 480 - protein, 10 aa, synthetic construct
QQYNQWPRYT

SEQ ID NO: 481 - protein, 123 aa, synthetic construct
EVQLVQSGAEVKKPGESLKISCKASGYNFNTYWIGWVRQMPGKGLEWMGIIYPGDSDTRYSPSFQGQVTISADKSISTAFLQWSSLKASDTAMYYCARLPYDSSGSSLPNDYWGQGTLVTVSS

SEQ ID NO: 482 - protein, 8 aa, synthetic construct
GYNFNTYW

SEQ ID NO: 483 - protein, 8 aa, synthetic construct
IYPGDSDT

SEQ ID NO: 484 - protein, 16 aa, synthetic construct
ARLPYDSSGSSLPNDY

SEQ ID NO: 485 - protein, 109 aa, synthetic construct
QSVVTQPPSASGTPGQRVTISCSGSSSNIGSNYVYWYQQLPGTAPKLLIYGNNQRPSGVPDRLSGSKSGTSASLAISGLRSEDEADYYCATWDDSLSGPVFGGGTKLTV

SEQ ID NO: 486 - protein, 8 aa, synthetic construct
SSNIGSNY

SEQ ID NO: 487 - skipped

SEQ ID NO: 488 - protein, 11 aa, synthetic construct
ATWDDSLSGPV

SEQ ID NO: 489 - protein, 124 aa, synthetic construct
EVQLVESGGGLVLPGGSLRLSCAASGFTFSSYWMNWVRQTPGKGLEWVANIKQDGTDKYYVDSVKGRFTISRDNAKNSLFLQMTSLRAEDTAVYYCARYYHDNGRYYSYFFDLWGQGTLVTVSS

SEQ ID NO: 490 - protein, 8 aa, synthetic construct
GFTFSSYW

SEQ ID NO: 491 - protein, 8 aa, synthetic construct
IKQDGTDK

SEQ ID NO: 492 - protein, 17 aa, synthetic construct
ARYYHDNGRYYSYFFDL

SEQ ID NO: 493 - protein, 113 aa, synthetic construct
DTVLTQSPDSLAVSLGERATINCKSSQTLLYRSNNKNYLGWYKQKPGQPPKLLIYWASIRESGVPDRISGSGSGTDFTLTINSLQAEDVAVYYCQQYYSSPPTFGQGTKVEIK

SEQ ID NO: 494 - protein, 12 aa, synthetic construct
QTLLYRSNNKNY

SEQ ID NO: 495 - skipped

SEQ ID NO: 496 - protein, 9 aa, synthetic construct
QQYYSSPPT

SEQ ID NO: 497 - protein, 226 aa, synthetic construct
MESTTSGFLGPLLVLQAGFFLLTRILTIPQSLDSWWTSLNFLGGAPTCPGQNSQSPTSNHSPTSCPPICPGYRWMCLRRFIIFLFILLLCLIFLLVLLDYQGMLPVCPLLPGTSTTSTGPCKTCTIPAQGTSMFPSCCCTKPSDGNCTCIPIPSSWAFARFLWEWASVRFSWLSLLVPFVQWFAGLSPTVWLSVIWMMWYWGPSLYNILSPFLPLLPIFFCLWVYI